European Patent Specification EP 3 896 452 B1, published May 10, 2023. Title: METHOD FOR ASSISTING PREDICTION OF EXACERBATION OF RESPIRATORY INFECTION AND REAGENT KIT. Applicant: NATIONAL CENTER FOR GLOBAL HEALTH AND MEDICINE SYSMEX CORPORATION. The sequence listing filed with the application follows.

SEQUENCE LISTING (12 sequences)

SEQ ID NO: 1 - protein, 200 aa, Homo sapiens
MKLDMTGDCMPVLVLMAAVLTVTGAVPVARLRGALPDARGCHIAQFKSLSPQELQAFKRAKDALEESLLLKDCKCRSRLFPRTWDLRQLQVRERPVALEAELALTLKVLEATADTDPALGDVLDQPLHTLHHILSQLRACIQPQPTAGPRTRGRLHHWLHRLQEAPKKESPGCLEASVTFNLFRLLTRDLNCVASGDLCV

SEQ ID NO: 2 - protein, 200 aa, Homo sapiens
MKLDMTGDCMPVLVLMAAVLTVTGAVPVARLRGALPDARGCHIAQFKSLSPQELQAFKRAKDALEESLLLKDCRCRSRLFPRTWDLRQLQVRERPVALEAELALTLKVLEATADTDPALGDVLDQPLHTLHHILSQLRACIQPQPTAGPRTRGRLHHWLHRLQEAPKKESPGCLEASVTFNLFRLLTRDLNCVASGDLCV

SEQ ID NO: 3 - protein, 124 aa, Mus musculus
EVQLVESGGDLVKPGGSLKLSCAASGFTFSSYGMSWVRHIPDKRLEWVATITGGGSYTYYPDGVKGRFTISRDNAKNTLYLQMSSLKSEDTAMYYCARRGDYGSNYLYWYFDVWGAGTTVTVSS

SEQ ID NO: 4 - protein, 108 aa, Mus musculus
DIVLTQSPASLAVSLGQRATISYRASKSVSTSGYSYMHWNQQKPGQPPRLLIYLVSNLESGVPARFSGSGSGTDFTLNIHPVEEEDAATYYCQHIRELTRSEGGPSWK

SEQ ID NO: 5 - protein, 120 aa, Mus musculus
EVKLVESGGGLVQPGGSLKLSCATSGFTFSDYYMYWVRQTPEKRLEWVAYISNGGGSTNYPDTVKGRFTISRDNAKNTLYLQMSRLKSEDTAMYYCARPSLLRSAWFAYWGQGTLVTVSA

SEQ ID NO: 6 - protein, 108 aa, Mus musculus; identical to SEQ ID NO: 4

SEQ ID NO: 7 - protein, 117 aa, Mus musculus
EVQLQQSGAELVKPGASVKLSCTASGFNIKDTYIHWVKQRPEQGLEWIGRIDPANGNTKYDPKFQGKATITADTSSNTAYLQLSSLTSEDTAVYFCAPYGYDYFDYWGQGTTLTVSS

SEQ ID NO: 8 - protein, 108 aa, Mus musculus; identical to SEQ ID NO: 4

SEQ ID NO: 9 - protein, 117 aa, Mus musculus; identical to SEQ ID NO: 7

SEQ ID NO: 10 - protein, 108 aa, Mus musculus; identical to SEQ ID NO: 4

SEQ ID NO: 11 - protein, 117 aa, Mus musculus
EVQLQQSGAELVKPGASVTLSCTASGFNIRDTYIHWVKQRPEQGLEWIGRIDPANGNIKYDPKFQGKATITADTSSNTAYLQLSSLTSEDTAVYYCTPYGYDYFDYWGQGTTLTVSS

SEQ ID NO: 12 - protein, 108 aa, Mus musculus; identical to SEQ ID NO: 4